European Patent Application EP 4 488 261 A1, published January 8, 2025. Title: Amino lipid compound, preparation method therefor, composition thereof and use thereof. Applicant: SHENZHEN SHENXIN BIOTECHNOLOGY CO., LTD. The sequence listing filed with the application follows.

SEQUENCE LISTING (1 sequence)

SEQ ID NO: 1 - RNA, 4234 nt, synthetic construct
  source 1..4234: mol_type = other RNA
  misc_feature 1..2: note = cap G1G2 = m7G+-5'-ppp-5'-Gm2'-3'-p- [m7 = 7-CH3; m2' = 2'-O-CH3; -ppp- = -PO2H-O-PO2H-O-PO2H)-; -p- = -PO2H-]
ggggaaagctttaatacgactcactataggacagatcgcctggagacgccatccacgctgttttgacctccatagaagacaccgggaccgatccagcctccgcggccgggaacggtgcattggaacgcggattccccgtgccaagagtgacgtaagtaccgcagtcaccgtccttgacacgggatccgccaccatgttcgtgttcctggtgctgctgcctctggtgtccagccagtgtgtgaacctgaggaccagaacacagctgcctccagcctacaccaacagctttaccagaggcgtgtactaccccgacaaggtgttcagatccagcgtgctgcactctacccaggacctgttcctgcctttcttcagcaacgtgacctggttccacgccatccacgtgtccggcaccaatggcaccaagagattcgacaaccccgtgctgcccttcaacgacggggtgtactttgccagcatcgagaagtccaacatcatcagaggctggatcttcggcaccacactggacagcaagacccagagcctgctgatcgtgaacaacgccaccaacgtggtcatcaaagtgtgcgagttccagttctgcaacgaccccttcctggacgtctactaccacaagaacaacaagagctggatggaaagcggcgtgtacagcagcgccaacaactgcaccttcgagtacgtgtcccagcctttcctgatggacctggaaggcaagcagggcaacttcaagaacctgcgcgagttcgtgtttaagaacatcgacggctacttcaagatctacagcaagcacacccctatcaacctcgtgcgggatctgcctcagggcttctctgctctggaacccctggtggatctgcccatcggcatcaacatcacccggtttcagacactgctggccctgcacagaagctacctgacacctggcgatagcagcagcggactgacagctggtgccgccgcttactatgtgggctacctgcagcctagaaccttcctgctgaagtacaacgagaacggcaccatcaccgacgccgtggattgtgctctggaccctctgagcgagacaaagtgcaccctgaagtccttcaccgtggaaaagggcatctaccagaccagcaacttccgggtgcagcccaccgaatccatcgtgcggttccccaatatcaccaatctgtgccccttcggcgaggtgttcaatgccaccagattcgcctctgtgtacgcctggaaccggaagcggatcagcaattgcgtggccgactactccgtgctgtacaactccgccagcttcagcaccttcaagtgctacggcgtgtcccctaccaagctgaacgacctgtgcttcacaaacgtgtacgccgacagcttcgtgatccggggagatgaagtgcggcagattgcccctggacagacaggcaacatcgccgactacaactacaagctgcccgacgacttcaccggctgtgtgattgcctggaacagcaacaacctggactccaaagtcggcggcaactacaattaccggtacaggctgttccggaagtccaatctgaagcccttcgagcgggacatctccaccgagatctatcaggccggcagcaagccttgtaacggcgtggaaggcttcaactgctacttcccactgcagtcctacggctttcagcccacaaatggcgtgggctatcagccctacagagtggtggtgctgagcttcgaactgctgcatgcccctgccacagtgtgcggccctaagaaaagcaccaatctcgtgaagaacaaatgcgtgaacttcaacttcaacggcctgaccggcaccggcgtgctgacagagagcaacaagaagttcctgccattccagcagtttggccgggatatcgccgataccacagacgccgttagagatccccagacactggaaatcctggacatcaccccttgcagcttcggcggagtgtctgtgatcacccctggcaccaacaccagcaatcaggtggcagtgctgtaccagggcgtgaactgtaccgaagtgcccgtggccattcacgccgatcagctgacacctacatggcgggtgtactccaccggcagcaatgtgtttcagaccagagccggctgtctgatcggagccgagcacgtgaacaatagctacgagtgcgacatccccatcggcgctggaatctgcgccagctaccagacacagacaaacagccggcggagagccagaagcgtggccagccagagcatcattgcctacacaatgtctctgggcgccgagaacagcgtggcctactccaacaactctatcgctatccccaccaacttcaccatcagcgtgaccacagagatcctgcctgtgtccatgaccaagaccagcgtggactgcaccatgtacatctgcggcgattccaccgagtgctccaacctgctgctgcagtacggcagcttctgcacccagctgaatagagccctgacagggatcgccgtggaacaggacaagaacacccaagaggtgttcgcccaagtgaagcagatctacaagacccctcctatcaaggacttcggcggcttcaatttcagccagattctgcccgatcctagcaagcccagcaagcggagcttcatcgaggacctgctgttcaacaaagtgacactggccgacgccggcttcatcaagcagtatggcgattgtctgggcgacattgccgccagggatctgatttgcgcccagaagtttaacggactgacagtgctgcctcctctgctgaccgatgagatgatcgcccagtacacatctgccctgctggccggcacaatcacaagcggctggacatttggagcaggcgccgctctgcagatcccctttgctatgcagatggcctaccggttcaacggcatcggagtgacccagaatgtgctgtacgagaaccagaagctgatcgccaaccagttcaacagcgccatcggcaagatccaggacagcctgagcagcacagcaagcgccctgggaaagctgcagaacgtggtcaaccagaatgcccaggcactgaacaccctggtcaagcagctgtcctccaacttcggcgccatcagctctgtgctgaacgatatcctgagcagactggaccctcctgaggccgaggtgcagatcgacagactgatcacaggcagactgcagagcctccagacatacgtgacccagcagctgatcagagccgccgagattagagcctctgccaatctggccgccaccaagatgtctgagtgtgtgctgggccagagcaagagagtggacttttgcggcaagggctaccacctgatgagcttccctcagtctgcccctcacggcgtggtgtttctgcacgtgacatatgtgcccgctcaagagaagaatttcaccaccgctccagccatctgccacgacggcaaagcccactttcctagagaaggcgtgttcgtgtccaacggcacccattggttcgtgacacagcggaacttctacgagccccagatcatcaccaccgacaacaccttcgtgtctggcaactgcgacgtcgtgatcggcattgtgaacaataccgtgtacgaccctctgcagcccgagctggacagcttcaaagaggaactggacaagtactttaagaaccacacaagccccgacgtggacctgggcgatatcagcggaatcaatgccagcgtcgtgaacatccagaaagagatcgaccggctgaacgaggtggccaagaatctgaacgagagcctgatcgacctgcaagaactggggaagtacgagcagtacatcaagtggccctggtacatctggctgggctttatcgccggactgattgccatcgtgatggtcacaatcatgctgtgttgcatgaccagctgctgtagctgcctgaagggctgttgtagctgtggcagctgctgcaagttcgacgaggacgattctgagcccgtgctgaagggcgtgaaactgcactacacatgatgaggtacccgggtggcatccctgtgacccctccccagtgcctctcctggccctggaagttgccactccagtgcccaccagccttgtcctaataaaattaagttgcatcgggcccaaaaaaaaaaaaaaaaaaaaaaaaaaaaaagcatatgactaaaaaaaaaaaaaaaaaaaaaaaaaaaaaaaaaaaaaaaaaaaaaaaaaaaaaaaaaaaaaaaaaaaaaa